European Patent Application EP 4 781 828 A1, published July 29, 2026. Title: Non-sporulating, non-lysing Bacillus thuringiensis strain and its use as biopesticide. Applicant: Institut national de recherche pour l agriculture, l alimentation et l environnement. The sequence listing filed with the application follows.

SEQUENCE LISTING (12 sequences)

SEQ ID NO: 1 - protein, 318 aa, Bacillus thuringiensis
  VARIANT 6: note = T or V
  VARIANT 11: note = K or N
  VARIANT 12: note = I or T
  VARIANT 30: note = S or T
  VARIANT 34: note = G or R
  VARIANT 48: note = A or T
  VARIANT 64: note = S or T
  VARIANT 65: note = G or S
  VARIANT 75: note = H or N
  VARIANT 172: note = L or P
  VARIANT 228: note = D or E
  VARIANT 232: note = D or N
  VARIANT 242: note = P or S
  VARIANT 251: note = K or Q
  VARIANT 255: note = I or V
  VARIANT 257: note = K or R
  VARIANT 263: note = A or T
  VARIANT 273: note = D or N
  VARIANT 276: note = D or N
  VARIANT 277: note = K or R
  VARIANT 278: note = I or V
  VARIANT 290: note = L or Q
  VARIANT 295: note = I or V
  VARIANT 310: note = A or T
MTVFNXKEINXXPFESNIIPKGNRNRPAYXMNPXYITIHTTANQNAGXDARAHARYVNNGGGSXXVSWHFTVDDXRIVQHLPLNENGWHAGDGNGAGNRSSIGIEICENRDGNFEKALTHAAGLVKFLMAHLGLKIGNVVSHQHWSGKNCPRPIFNRPGGFEGFKRMIEDSXNDMVVENHNKDAGTQGLGIAYMEGVNINLRRGPSTSSDVIRKLNKPESYIVWEERXGWLXLGNSWVKYDXSYIYFARRXTSNXGXLVVVDXNELWVYGSAXWNXXXKTVKKGEAFTIXDELQXNGSNMYKCKYFYITXNSQFVYVK

SEQ ID NO: 2 - DNA, 30 bp, Bacillus thuringiensis
  source 1..30: mol_type = genomic DNA
  variation 4: note = A or T or C or G
  variation 5: note = A or T or C or G
  variation 6: note = A or T or C or G
  variation 7: note = A or T or C or G
  variation 10: note = A or T or C or G
  variation 12: note = A or T or C or G
  variation 13: note = A or T or C or G
  variation 17: note = A or T or C or G
  variation 18: note = A or T or C or G
  variation 22: note = A or T or C or G
  variation 24: note = A or T or C or G
  variation 26: note = A or T or C or G
ttcnnnnatngnngaanntatntntncttt

SEQ ID NO: 3 - protein, 318 aa, Bacillus thuringiensis
MTVFNTKEINNTPFESNIIPKGNRNRPAYSMNPRYITIHTTANQNAGTDARAHARYVNNGGGSSSVSWHFTVDDNRIVQHLPLNENGWHAGDGNGAGNRSSIGIEICENRDGNFEKALTHAAGLVKFLMAHLGLKIGNVVSHQHWSGKNCPRPIFNRPGGFEGFKRMIEDSLNDMVVENHNKDAGTQGLGIAYMEGVNINLRRGPSTSSDVIRKLNKPESYIVWEEREGWLNLGNSWVKYDSSYIYFARRQTSNIGKLVVVDTNELWVYGSANWNDKIKTVKKGEAFTIQDELQVNGSNMYKCKYFYITTNSQFVYVK

SEQ ID NO: 4 - protein, 318 aa, Bacillus thuringiensis
MTVFNVKEINKIPFESNIIPKGNRNRPAYTMNPRYITIHTTANQNAGADARAHARYVNNGGGSSGVSWHFTVDDHRIVQHLPLNENGWHAGDGNGAGNRSSIGIEICENRDGNFEKALTHAAGLVKFLMAHLGLKIGNVVSHQHWSGKNCPRPIFNRPGGFEGFKRMIEDSLNDMVVENHNKDAGTQGLGIAYMEGVNINLRRGPSTSSDVIRKLNKPESYIVWEEREGWLNLGNSWVKYDSSYIYFARRQTSNIGKLVVVDTNELWVYGSANWNDKIKTVKKGEAFTIQDELQVNGSNMYKCKYFYITANSQFVYVK

SEQ ID NO: 5 - protein, 318 aa, Bacillus thuringiensis; identical to SEQ ID NO: 3

SEQ ID NO: 6 - protein, 318 aa, Bacillus thuringiensis
MTVFNTKEINNTPFESNIIPKGNRNRPAYSMNPRYITIHTTANQNAGADARAHARYVNNGGGSSGVSWHFTVDDNRIVQHLPLNENGWHAGDGNGAGNRSSIGIEICENRDGNFEKALTHAAGLVKFLMAHLGLKIGNVVSHQHWSGKNCPRPIFNRPGGFEGFKRMIEDSLNDMVVENHNKDAGTQGLGIAYMEGVNINLRRGPSTSSDVIRKLNKPESYIVWEEREGWLNLGNSWVKYDSSYIYFARRQTSNIGKLVVVDTNELWVYGSANWNDKIKTVKKGEAFTIQDELQVNGSNMYKCKYFYITTNSQFVYVK

SEQ ID NO: 7 - protein, 318 aa, Bacillus thuringiensis; identical to SEQ ID NO: 4

SEQ ID NO: 8 - protein, 318 aa, Bacillus thuringiensis; identical to SEQ ID NO: 3

SEQ ID NO: 9 - protein, 318 aa, Bacillus thuringiensis
MTVFNVKEINKIPFESNIIPKGNRNRPAYTMNPRYITIHTTANQNAGADARAHARYVNNGGGSSGVSWHFTVDDHRIVQHLPLNENGWHAGDGNGAGNRSSIGIEICENRDGNFEKALTHAAGLVKFLMAHLGLKIGNVVSHQHWSGKNCPRPIFNRPGGFEGFKRMIEDSLNDMVVENHNKDAGTQGLGIAYMEGVNINLRRGPSTSSDVIRKLNKPESYIVWEEREGWLNLGNSWVKYDSSYIYFARRQTSNIGKLVVVDTNELWVYGSANWNDKIKTVKKGEAFTIQDELQVNGSNMYKCKYFYITTNSQFVYVK

SEQ ID NO: 10 - protein, 318 aa, Bacillus thuringiensis; identical to SEQ ID NO: 3

SEQ ID NO: 11 - protein, 318 aa, Bacillus thuringiensis
MTVFNVKEINNTPFESNIIPKGNRNRPAYSMNPGYITIHTTANQNAGADARAHARYVNNGGGSTGVSWHFTVDDNRIVQHLPLNENGWHAGDGNGAGNRSSIGIEICENRDGNFEKALTHAAGLVKFLMAHLGLKIGNVVSHQHWSGKNCPRPIFNRPGGFEGFKRMIEDSPNDMVVENHNKDAGTQGLGIAYMEGVNINLRRGPSTSSDVIRKLNKPESYIVWEERDGWLDLGNSWVKYDPSYIYFARRKTSNVGRLVVVDANELWVYGSADWNNRVKTVKKGEAFTILDELQINGSNMYKCKYFYITANSQFVYVK

SEQ ID NO: 12 - protein, 318 aa, Bacillus thuringiensis; identical to SEQ ID NO: 4